European Patent Specification EP 3 312 278 B1, published December 4, 2024. Title: METHOD FOR EXPRESSING PROTEINS. Applicant: NATIONAL UNIVERSITY CORPORATION NAGOYA UNIVERSITY. The sequence listing filed with the application follows.

SEQUENCE LISTING (50 sequences)

SEQ ID NO: 1 - protein, 4 aa, Artificial Sequence
  tag sequence
  MISC_FEATURE (3)..(3): any amino acid
  MISC_FEATURE (4)..(4): any amino acid
SKXX

SEQ ID NO: 2 - protein, 4 aa, Artificial Sequence
  tag sequence
  MISC_FEATURE (4)..(4): any amino acid
SKIX

SEQ ID NO: 3 - protein, 4 aa, Artificial Sequence
  tag sequence
SKIK

SEQ ID NO: 4 - DNA, 12 bp, Artificial Sequence
  tag sequence
tctaaaataaaa

SEQ ID NO: 5 - DNA, 12 bp, Artificial Sequence
  tag sequence
tcgaagatcaag

SEQ ID NO: 6 - DNA, 43 bp, Artificial Sequence
  primer
ttaagaaggagatatacatatggaggtccagctgcaacagtcc

SEQ ID NO: 7 - DNA, 49 bp, Artificial Sequence
  primer
gagctgggcgctcccaccaccgcctggaatgggcacatgcagatctttg

SEQ ID NO: 8 - DNA, 47 bp, Artificial Sequence
  primer
taataatctagaaggagatatcatatggatgttttgatgacccaaac

SEQ ID NO: 9 - DNA, 43 bp, Artificial Sequence
  primer
ctgggcgctcccaccaccgccacactctttcctgttgaagctc

SEQ ID NO: 10 - DNA, 33 bp, Artificial Sequence
  primer
ggcggtggtgggagcgcccagctcgaaaaggag

SEQ ID NO: 11 - DNA, 41 bp, Artificial Sequence
  primer
tgatatctccttctagattattaagcgtaatctggaacatc

SEQ ID NO: 12 - DNA, 34 bp, Artificial Sequence
  primer
ggcggtggtgggagcgcccagctcaagaagaagc

SEQ ID NO: 13 - DNA, 30 bp, Artificial Sequence
  primer
tcgtcgtccttgtagtcggaaccgcccttc

SEQ ID NO: 14 - DNA, 52 bp, Artificial Sequence
  primer
ccgactacaaggacgacgatgacaaataataagatccggctgctaacaaagc

SEQ ID NO: 15 - DNA, 22 bp, Artificial Sequence
  primer
catatgtatatctccttcttaa

SEQ ID NO: 16 - DNA, 40 bp, Artificial Sequence
  primer
aggagatatacatatgtctaaaataaaagaggtccagctg

SEQ ID NO: 17 - DNA, 44 bp, Artificial Sequence
  primer
gtcatcaaaacatcttttattttagacatatgatatctccttct

SEQ ID NO: 18 - DNA, 30 bp, Artificial Sequence
  primer
taaaataaaagatgttttgatgacccaaac

SEQ ID NO: 19 - DNA, 23 bp, Artificial Sequence
  primer
tagacatatgtatatctccttct

SEQ ID NO: 20 - DNA, 33 bp, Artificial Sequence
  T7 tag
atggctagcatgactggtggacagcaaatgggt

SEQ ID NO: 21 - protein, 11 aa, Artificial Sequence
  T7 tag
MASMTGGQQMG

SEQ ID NO: 22 - DNA, 25 bp, Artificial Sequence
  primer
atctcgatcccgcgaaattaatacg

SEQ ID NO: 23 - DNA, 24 bp, Artificial Sequence
  primer
tccggatatagttcctcctttcag

SEQ ID NO: 24 - DNA, 28 bp, Artificial Sequence
  primer
ttttttcggtaccaagcttaatattccc

SEQ ID NO: 25 - DNA, 27 bp, Artificial Sequence
  primer
taactgatcctagagggccgcatcatg

SEQ ID NO: 26 - DNA, 43 bp, Artificial Sequence
  primer
taagcttggtaccgaaaaaaatggatgtcgtgatgacccagac

SEQ ID NO: 27 - DNA, 42 bp, Artificial Sequence
  primer
ggccctctaggatcagttaagcgtaatctggaacatcgtatg

SEQ ID NO: 28 - DNA, 50 bp, Artificial Sequence
  primer
taagcttggtaccgaaaaaaatgtctaaaataaaagatgtcgtgatgacc

SEQ ID NO: 29 - protein, 4 aa, Artificial Sequence
  tag sequence
  MISC_FEATURE (3)..(3): any amino acid
  MISC_FEATURE (4)..(4): any amino acid
AKXX

SEQ ID NO: 30 - protein, 4 aa, Artificial Sequence
  tag sequence
  MISC_FEATURE (3)..(3): any amino acid
  MISC_FEATURE (4)..(4): any amino acid
KKXX

SEQ ID NO: 31 - protein, 4 aa, Artificial Sequence
  tag sequence
SKII

SEQ ID NO: 32 - protein, 4 aa, Artificial Sequence
  tag sequence
SKKK

SEQ ID NO: 33 - protein, 4 aa, Artificial Sequence
  tag sequence
AKIK

SEQ ID NO: 34 - protein, 4 aa, Artificial Sequence
  tag sequence
AKII

SEQ ID NO: 35 - protein, 4 aa, Artificial Sequence
  tag sequence
KKKK

SEQ ID NO: 36 - DNA, 12 bp, Artificial Sequence
  tag sequence
tctaaaattatt

SEQ ID NO: 37 - DNA, 12 bp, Artificial Sequence
  tag sequence
tctaaaaaaaaa

SEQ ID NO: 38 - DNA, 12 bp, Artificial Sequence
  tag sequence
gcaaaaattaaa

SEQ ID NO: 39 - DNA, 12 bp, Artificial Sequence
  tag sequence
gcaaaaattatt

SEQ ID NO: 40 - DNA, 12 bp, Artificial Sequence
  tag sequence
aaaaaaaaaaaa

SEQ ID NO: 41 - DNA, 32 bp, Artificial Sequence
  primer
atatgaaaaaaaaaaaagaccctatgctgacc

SEQ ID NO: 42 - DNA, 33 bp, Artificial Sequence
  primer
agggtcttttttttttttcatatgtatatctcc

SEQ ID NO: 43 - DNA, 32 bp, Artificial Sequence
  primer
atatggcaaaaattaaagaccctatgctgacc

SEQ ID NO: 44 - DNA, 33 bp, Artificial Sequence
  primer
agggtctttaatttttgccatatgtatatctcc

SEQ ID NO: 45 - DNA, 32 bp, Artificial Sequence
  primer
atatgtctaaaaaaaaagaccctatgctgacc

SEQ ID NO: 46 - DNA, 33 bp, Artificial Sequence
  primer
agggtctttttttttagacatatgtatatctcc

SEQ ID NO: 47 - DNA, 32 bp, Artificial Sequence
  primer
atatggcaaaaattattgaccctatgctgacc

SEQ ID NO: 48 - DNA, 33 bp, Artificial Sequence
  primer
agggtcaataatttttgccatatgtatatctcc

SEQ ID NO: 49 - DNA, 32 bp, Artificial Sequence
  primer
atatgtctaaaattattgaccctatgctgacc

SEQ ID NO: 50 - DNA, 33 bp, Artificial Sequence
  primer
agggtcaataattttagacatatgtatatctcc